European Patent Specification EP 3 516 394 B1, published June 21, 2023. Title: Mycobacterium tuberculosis Proteins in Diagnostic Assays and Devices for Tuberculosis Detection and Diagnosis. Applicant: Nguyen, Hiep-Hoa T. The sequence listing filed with the application follows.

SEQUENCE LISTING (16 sequences)

SEQ ID NO: 1 - protein, 144 aa, Mycobacterium tuberculosis
MADKTTQTIYIDADPGEVMKAIADIEAYPQWISEYKEVEILEADDEGYPKRARMLMDAAIFKDTLIMSYEWPEDRQSLSWTLESSSLLKSLEGTYRLAPKGSGTEVTYELAVDLAVPMIGMLKRKAERRLIDGALKDLKKRVEG

SEQ ID NO: 2 - DNA, 435 bp, Mycobacterium tuberculosis
gtggcggacaagacgacacagacgatttacatcgacgcggatccaggcgaggtgatgaaggcgatcgccgacatcgaagcctacccgcaatggatttcggagtataaggaagtcgagatcctagaggccgacgacgagggctacccgaaacgagcgcgaatgttgatggacgcagccatcttcaaagacaccttgatcatgtcctacgagtggccggaagaccgccaatcgcttagctggactctcgaatccagctcgctgctaaagtccctcgaaggcacgtatcgcttggcgcccaagggttctggcactgaggtcacctacgagcttgccgtcgaccttgctgtccccatgatcgggatgctcaagcgtaaggcggaacgcaggttgatagacggcgcgttgaaggatctgaagaaacgagtcgagggctga

SEQ ID NO: 3 - protein, 129 aa, Mycobacterium tuberculosis
MNLRRHQTLTLRLLAASAGILSAAAFAAPAQANPVDDAFIAALNNAGVNYGDPVDAKALGQSVCPILAEPGGSFNTAVASVVARAQGMSQDMAQTFTSIAISMYCPSVMADVASGNLPALPDMPGLPGS

SEQ ID NO: 4 - DNA, 390 bp, Mycobacterium tuberculosis
atgaacctacggcgccatcagaccctgacgctgcgactgctggcggcatccgcgggcattctcagcgccgcggccttcgccgcgccagcacaggcaaaccccgtcgacgacgcgttcatcgccgcgctgaacaatgccggcgtcaactacggcgatccggtcgacgccaaagcgctgggtcagtccgtctgcccgatcctggccgagcccggcgggtcgtttaacaccgcggtagccagcgttgtggcgcgcgcccaaggcatgtcccaggacatggcgcaaaccttcaccagtatcgcgatttcgatgtactgcccctcggtgatggcagacgtcgccagcggcaacctgccggccctgccagacatgccggggctgcccgggtcctag

SEQ ID NO: 5 - protein, 262 aa, Mycobacterium tuberculosis
MSSESDAANTEPEVLVEQRDRILIITINRPKAKNAVNAAVSRGLADAMDQLDGDAGLSVAILTGGGGSFCAGMDLKAFARGENVVVEGRGLGFTERPPTKPLIAAVEGYALAGGTELALAADLIVAARDSAFGIPEVKRGLVAGGGGLLRLPERIPYAIAMELALTGDNLPAERAHELGLVNVLAEPGTALDAAIALAEKITANGPLAVVATKRIITESRGWSPDTMFAEQMKILVPVFTSNDAKEGAIAFAERRRPRWTGT

SEQ ID NO: 6 - DNA, 789 bp, Mycobacterium tuberculosis
atgagcagcgaaagcgacgcagccaacaccgaacctgaggttctggtagaacagcgggatcggattttgatcatcacgatcaaccgcccgaaagccaagaacgcggtcaacgccgcagtcagccggggcttggccgatgcgatggatcagcttgacggcgatgccggcctgtcggtggcaatcctgaccggtgggggcggttcgttctgcgcgggcatggacctcaaggcgttcgcccggggcgagaatgtcgtcgtcgaaggtcgcggccttggctttaccgaacgtccgccgaccaagccgctcattgctgcggtggaaggctacgcgttggcgggtggcaccgagctggcgcttgctgccgacctgatcgtggcggccagggattcggcgttcgggattcctgaagtcaagcggggtctggttgccggcggcgggggattgctgcggttgccggagcgcatcccgtatgcgatagccatggagttggcgctgaccggtgacaacctaccggccgaacgcgcgcacgagctggggctcgtcaacgttttggccgagccggggaccgccctcgatgctgcgatcgcgttggcggagaagatcaccgccaatgggccgctggcggtggtggccaccaagcggattatcaccgagtcgcgtgggtggagtcccgacactatgttcgctgagcagatgaagatcctggtgccggtgttcacctccaacgacgcgaaggaaggtgcgatcgcgttcgccgagaggcgccggccccgttggacgggcacctag

SEQ ID NO: 7 - protein, 186 aa, Mycobacterium tuberculosis
MSDALDEGLVQRIDARGTIEWSETCYRYTGAHRDALSGEGARRFGGRWNPPLLFPAIYLADSAQACMVEVERAAQAASTTAEKMLEAAYRLHTIDVTDLAVLDLTTPQAREAVGLENDDIYGDDWSGCQAVGHAAWFLHMQGVLVPAAGGVGLVVTAYEQRTRPGQLQLRQSVDLTPALYQELRAT

SEQ ID NO: 8 - DNA, 561 bp, Mycobacterium tuberculosis
gtgagcgatgccctcgatgaagggctcgtccagcgtatcgacgcacgcggaacaattgagtggtcggaaacgtgctaccggtataccggcgcgcaccgtgacgccttgtccggtgagggcgcgcgcagattcggaggcaggtggaatccgccgctgctctttccggcgatctatcttgctgattccgcccaagcctgcatggttgaggtggaacgggcggcgcaagcggcttcaacgaccgcagagaagatgctcgaggcggcctaccgactacacacgatcgacgtcacggacctggccgtcctcgatctgacaaccccgcaagctcgggaagccgtggggctcgagaacgacgacatctatggcgacgactggtcagggtgccaggcggtcggacatgcggcctggttcttgcacatgcaaggtgtcctcgtgccggcggcgggcggtgtcggcctcgttgtcaccgcgtatgaacagcgaactcggccgggccaactacaactgcgacaaagcgtcgatctgacgcctgctctttaccaagaacttcgagccacgtag

SEQ ID NO: 9 - protein, 200 aa, Mycobacterium tuberculosis
MSPSPSALLADHPDRIRWNAKYECADPTEAVFAPISWLGDVLQFGVPEGPVLELACGRSGTALGLAAAGRCVTAIDVSDTALVQLELEATRRELADRLTLVHADLCSWQSGDGRFALVLCRLFWHPPTFRQACEAVAPGGVVAWEAWRRPIDVARDTRRAEWCLKPGQPESELPAGFTVIRVVDTDGSEPSRRIIAQRSL

SEQ ID NO: 10 - DNA, 603 bp, Mycobacterium tuberculosis
atgagtccgtctccatcggccctgctcgccgaccacccggaccgcattcgttggaacgcgaaatacgagtgcgctgaccccacggaggcggtatttgcgcccatatcctggctcggcgacgtgctgcagttcggggtgccagaagggccggttctggaactggcgtgcggtcggtccggcaccgcgctggggctagccgcggcgggccgctgcgtgactgcgatcgacgtttccgataccgcgttggttcagctcgagctcgaagcgacccgacgggaattggccgatcgcctcacactggtgcacgccgatctctgctcctggcagtcgggggatggacgctttgctctggtactttgccgactattctggcatccgcccacttttcgccaggcttgcgaggctgtggcgccgggcggtgtagtggcgtgggaggcatggcggcggcccatcgatgtcgctcgggatacccgtcgagccgaatggtgcttgaagccaggccagcccgagtctgaacttcccgccggcttcacggtgattcgggtggtcgacaccgatggttcagagccgtcgcggcgcatcatcgcccaacggtcactgtga

SEQ ID NO: 11 - protein, 100 aa, Mycobacterium tuberculosis
MCSGPKQGLTLPASVDLEKETVITGRVVDGDGQAVGGAFVRLLDSSDEFTAEVVASATGDFRFFAAPGSWTLRALSAAGNGDAVVQPSGAGIHEVDVKIT

SEQ ID NO: 12 - DNA, 303 bp, Mycobacterium tuberculosis
atgtgctctggacccaagcaaggactgacattgccggccagcgtcgacctggaaaaagaaacggtgatcaccggccgcgtagtggacggtgacggccaggccgtgggcggcgcgttcgtgcggctgctggactcctccgacgagttcaccgcggaggtcgtcgcgtcggccaccggcgatttccggttcttcgccgcgcccggatcctggacgctgcgcgcgctgtcggcggccggcaacggcgacgcggtggtgcagccctcgggcgcgggcatccacgaggtagacgtcaagatcacctga

SEQ ID NO: 13 - protein, 146 aa, Mycobacterium tuberculosis
MSAYKTVVVGTDGSDSSMRAVDRAAQIAGADAKLIIASAYLPQHEDARAADILKDESYKVTGTAPIYEILHDAKERAHNAGAKNVEERPIVGAPVDALVNLADEEKADLLVVGNVGLSTIAGRLLGSVPANVSRRAKVDVLIVHTT

SEQ ID NO: 14 - DNA, 441 bp, Mycobacterium tuberculosis
atgagcgcctataagaccgtggtggtaggaaccgacggttcggactcgtcgatgcgagcggtagatcgcgctgcccagatcgccggcgcagacgccaagttgatcatcgcctcggcatacctacctcagcacgaggacgctcgcgccgccgacattctgaaggacgaaagctacaaggtgacgggcaccgccccgatctacgagatcttgcacgacgccaaggaacgagcgcacaacgccggtgcgaaaaacgtcgaggaacggccgatcgtcggcgccccggtcgacgcgttggtgaacctggccgatgaggagaaggcggacctgctggtcgtcggcaatgtcggtctgagcacgatcgcgggtcggctgctcggatcggtaccggccaatgtgtcacgccgggccaaggtcgacgtgctgatcgtgcacaccacctag

SEQ ID NO: 15 - protein, 232 aa, Mycobacterium tuberculosis
MHLMIPAEYISNVIYEGPRADSLYAADQRLRQLADSVRTTAESLNTTLDELHENWKGSSSEWMADAALRYLDWLSKHSRQILRTARVIESLVMAYEETLLRVVPPATIANNREEVRRLIASNVAGGKHSSNRRPRGTIRAVPGRKYPSNGPLSKLDPICAIEAAPMAGAAADPQERVGPRGRRGLAGQQQCRGRPGPSLRCSHDTPRFQMNQAFHTMVNMLLTCFACQEKPR

SEQ ID NO: 16 - DNA, 699 bp, Mycobacterium tuberculosis
atgcatctaatgatacccgcggagtatatctccaacgtaatatatgaaggtccgcgtgctgactcattgtatgccgccgaccagcgattgcgacaattagctgactcagttagaacgactgccgagtcgctcaacaccacgctcgacgagctgcacgagaactggaaaggtagttcatcggaatggatggccgacgcggctttgcggtatctcgactggctgtctaaacactcccgtcagattttgcgaaccgcccgcgtgatcgaatccctcgtaatggcctatgaggagacacttctgagggtggtacccccggcgactatcgccaacaaccgcgaggaggtgcgcaggctgatcgcgagcaacgtggccgggggtaaacactccagcaatcgcagacctcgaggcacaatacgagcagtaccgggccgaaaatatccaagcaatggaccgctatctaagttggacccgatttgcgctatcgaagctgccccgatggcgggagccgccgcagatccacaggagcgggtaggtccaagaggccggcgcggtcttgcaggccagcaacaatgccgcggtcgaccaggcccatcgcttcgctgctcgcacgacacaccgcggtttcagatgaatcaggcgtttcacaccatggtgaacatgttgctgacgtgttttgcatgtcaggagaaaccgagatga